European Patent Application EP 4 435 115 A1, published September 25, 2024. Title: Improved padlock probes for nucleic acid detection by Hyperbranched Rolling Circle Amplification. Applicant: FUNDACIÓN DEL SECTOR PÚBLICO ESTATAL CENTRO NACIONAL DE INVESTIGACIONES ONCOLÓGICAS CARLOS III (F.S.P. CNIO). The sequence listing filed with the application follows.

SEQUENCE LISTING (34 sequences)

SEQ ID NO: 1 - protein, 298 aa, synthetic construct
MAITKPLLAATLENIEDVQFPCLATPKIDGIRSVKQTQMLSRTFKPIRNSVMNRLLTELLPEGSDGEISIEGATFQDTTSAVMTGHKMYNAKFSYYWFDYVTDDPLKKYIDRVEDMKNYITVHPHILEHAQVKIIPLIPVEINNITELLQYERDVLSKGFEGVMIRKPDGKYKFGRSTLKEGILLKMKQFKDAEATIISMTALFKNTNTKTKDNFGYSKRSTHKSGKVEEDVMGSIEVDYDGVVFSIGTGFDADQRRDFWQNKESYIGKMVKFKYFEMGSKDCPRFPVFIGIRHEEDR

SEQ ID NO: 2 - protein, 572 aa, synthetic construct
MPRKMYSCDFETTTKVEDCRVWAYGYMNIEDHSEYKIGNSLDEFMAWVLKVQADLYFHNLKFDGAFIINWLERNGFKWSADGLPNTYNTIISRMGQWYMIDICLGYKGKRKIHTVIYDSLKKLPFPVKKIAKDFKLTVLKGDIDYHKERPVGYKITPEEYAYIKNDIQIIAEALLIQFKQGLDRMTAGSDSLKGFKDIITTKKFKKVFPTLSLGLDKEVRYAYRGGFTWLNDRFKEKEIGEGMVFDVNSLYPAQMYSRLLPYGEPIVFEGKYVWDEDYPLHIQHIRCEFELKEGYIPTIQIKRSRFYKGNEYLKSSGGEIADLWLSNVDLELMKEHYDLYNVEYISGLKFKATTGLFKDFIDKWTYIKTTSEGAIKQLAKLMLNSLYGKFASNPDVTGKVPYLKENGALGFRLGEEETKDPVYTPMGVFITAWARYTTITAAQACYDRIIYCDTDSIHLTGTEIPDVIKDIVDPKKLGYWAHESTFKRAKYLRQKTYIQDIYMKEVDGKLVEGSPDDYTDIKFSVKCAGMTDKIKKEVTFENFKVGFSRKMKPKPVQVPGGVVLVDDTFTIK

SEQ ID NO: 3 - protein, 685 aa, synthetic construct
MPRKMYSCDFETTTKVEDCRVWAYGYMNIEDHSEYKIGNSLDEFMAWVLKVQADLYFHNLKFDGAFIINWLERNGFKWSADGLPNTYNTIISRMGQWYMIDICLGYKGKRKIHTVIYDSLKKLPFPVKKIAKDFKLTVLKGDIDYHKERPVGYKITPEEYAYIKNDIQIIAEALLIQFKQGLDRMTAGSDSLKGFKDIITTKKFKKVFPTLSLGLDKEVRYAYRGGFTWLNDRFKEKEIGEGMVFDVNSLYPAQMYSRLLPYGEPIVFEGKYVWDEDYPLHIQHIRCEFELKEGYIPTIQIKRSRFYKGNEYLKSSGGEIADLWLSNVDLELMKEHYDLYNVEYISGLKFKATTGLFKDFIDKWTYIKTTSEGAIKQLAKLMLNSLYGKFASNPDVTGKVPYLKENGALGFRLGEEETKDPVYTPMGVFITAWARYTTITAAQACYDRIIYCDTDSIHLTGTEIPDVIKDIVDPKKLGYWAHESTFKRAKYLRQKTYIQDIYMKEVDGKLVEGSPDDYTDIKFSVKCAGMTDKIKKEVTFENFKVGFSRKMKPKPVQVPGGVVLVDDTFTIKGTGSGAWKEWLERKVGEGRARRLIEYFGSAGEVGKLVENAEVSKLLEVPGIGDEAVARLVPGYKTLRDAGLTPAEAERVLKRYGSVSKVQEGATPDELRELGLGDAKIARILG

SEQ ID NO: 4 - DNA, 15 bp, synthetic construct
  source 1..15: mol_type = other DNA
  variation 12..15: note = nucleobases bound by phosphorothioate linkages
tgtaaaacgacggcc

SEQ ID NO: 5 - DNA, 15 bp, synthetic construct
  source 1..15: mol_type = other DNA
  variation 12..15: note = nucleobases bound by phosphorothioate linkages
caggaaacagctatg

SEQ ID NO: 6 - DNA, 10 bp, synthetic construct
  source 1..10: mol_type = other DNA
  variation 7..10: note = nucleobases bound by phosphorothioate linkages
tgtaaaacga

SEQ ID NO: 7 - DNA, 10 bp, synthetic construct
  source 1..10: mol_type = other DNA
  variation 7..10: note = nucleobases bound by phosphorothioate linkages
aacagctatg

SEQ ID NO: 8 - DNA, 74 bp, synthetic construct
  source 1..74: mol_type = other DNA
aaagtcctaggttgaaaaaatgtaaaacgacggccgaattcatagctgtttcctgaaaaattatattttaatag

SEQ ID NO: 9 - DNA, 196 bp, synthetic construct
  source 1..196: mol_type = other DNA
taatacgactcactataggtaacatcactaggtttcaaactttacttgctttacatagaagttatttgactcctggtgattcttcttcaggttggacagctggtgctgcagcttattatgtgggttatcttcaacctaggacttttctattaaaatataatgaaaatggaaccattacagatgctgtagactgtgc

SEQ ID NO: 10 - DNA, 10 bp, synthetic construct
  source 1..10: mol_type = other DNA
  variation 7..10: note = nucleobases bound by phosphorothioate linkages
tgtaaaacga

SEQ ID NO: 11 - DNA, 10 bp, synthetic construct
  source 1..10: mol_type = other DNA
  variation 7..10: note = nucleobases bound by phosphorothioate linkages
aacagctatg

SEQ ID NO: 12 - RNA, 41 nt, synthetic construct
  source 1..41: mol_type = other RNA
taatttctactaagtgtagatatagaaaagtcctaggttga

SEQ ID NO: 13 - skipped

SEQ ID NO: 14 - DNA, 35 bp, synthetic construct
  source 1..35: mol_type = other DNA
caggaaacagctatgaattcggccgtcgttttaca

SEQ ID NO: 15 - DNA, 35 bp, synthetic construct; identical to SEQ ID NO: 14
  source 1..35: mol_type = other DNA
  variation 31..35: note = nucleobases bound by a phosphorothioate linkages

SEQ ID NO: 16 - DNA, 74 bp, synthetic construct
  source 1..74: mol_type = other DNA
tgcggtggacgatggaaaaatgtaaaacgacggccgaattcatagctgtttcctgaaaaaccgctagaagcatt

SEQ ID NO: 17 - DNA, 78 bp, synthetic construct
  source 1..78: mol_type = other DNA
agataacccacataaaaaaatgtaaaacgacggccgaattcatagctgtttcctgaaaaattatattttaatagaaaa

SEQ ID NO: 18 - DNA, 12 bp, synthetic construct
  source 1..12: mol_type = other DNA
gtcctaggttga

SEQ ID NO: 19 - DNA, 37 bp, synthetic construct
  source 1..37: mol_type = other DNA
aaagtcctaggttgaaaaaatgtaaaacgacggccga

SEQ ID NO: 20 - DNA, 38 bp, synthetic construct
  source 1..38: mol_type = other DNA
attcatagctgtttcctgaaaaattatattttaataga

SEQ ID NO: 21 - DNA, 21 bp, synthetic construct
  source 1..21: mol_type = other DNA
  variation 17..21: note = nucleobases bound by phosphorothioate linkages
gaattcggccgtcgttttaca

SEQ ID NO: 22 - DNA, 14 bp, synthetic construct
  source 1..14: mol_type = other DNA
caggaaacagctat

SEQ ID NO: 23 - DNA, 90 bp, synthetic construct
  source 1..90: mol_type = other DNA
aaagtcctaggttgaaaaaatgtaaaacgacggccgaattcatagctgtttcctgaaaaattatattttaatagaaaaaaaaaaaaaaaa

SEQ ID NO: 24 - DNA, 30 bp, synthetic construct
  source 1..30: mol_type = other DNA
  variation 16: note = N represents sequence B
tgcggtggacgatggnccgctagaagcatt

SEQ ID NO: 25 - DNA, 30 bp, synthetic construct
  source 1..30: mol_type = other DNA
  variation 16: note = N represents sequence B
aaagtcctaggttganttatattttaatag

SEQ ID NO: 26 - DNA, 46 bp, synthetic construct
  source 1..46: mol_type = other DNA
  variation 16: note = N represents sequence B
aaagtcctaggttganttatattttaatagaaaaaaaaaaaaaaaa

SEQ ID NO: 27 - DNA, 46 bp, synthetic construct
  source 1..46: mol_type = other DNA
  variation 16: note = N represents sequence B
agataacccacataanttatattttaatagaaaagtcctaggttga

SEQ ID NO: 28 - DNA, 41 bp, synthetic construct
  source 1..41: mol_type = other DNA
  variation 38..41: note = nucleobases bound by phosphorothioate linkages
aaagtcctaggttgaaaaaatgtaaaacgacggccgaattc

SEQ ID NO: 29 - DNA, 34 bp, synthetic construct
  source 1..34: mol_type = other DNA
atagctgtttcctgaaaaattatattttaataga

SEQ ID NO: 30 - DNA, 20 bp, synthetic construct
  source 1..20: mol_type = other DNA
  variation 17..20: note = nucleobases bound by phosphorothioate linkages
caggaaacagctatgaattc

SEQ ID NO: 31 - DNA, 14 bp, synthetic construct
  source 1..14: mol_type = other DNA
  variation 10..14: note = nucleobases bound by phosphorothioate linkages
gccgtcgttttaca

SEQ ID NO: 32 - DNA, 30 bp, synthetic construct; identical to SEQ ID NO: 25
  source 1..30: mol_type = other DNA
  variation 16: note = N represents sequence B

SEQ ID NO: 33 - RNA, 50 nt, synthetic construct
  source 1..50: mol_type = other RNA
caacatcctgggcaataagatggagtacaactacaacgcccacaatgtgt

SEQ ID NO: 34 - RNA, 50 nt, synthetic construct
  source 1..50: mol_type = other RNA
tccggcccctccatcgtccaccgcaaatgcttctaggcggactatgactt